European Patent Specification EP 3 448 884 B9, published July 26, 2023. Title: ENGINEERED MAMMALIAN CELLS FOR PRODUCTION OF RECOMBINANT PROTEINS. Applicant: Danmarks Tekniske Universitet. The sequence listing filed with the application follows.

SEQUENCE LISTING (24 sequences)

SEQ ID NO: 1 - DNA, 54 bp, Artificial Sequence
  DNA primer
ggaaaggacgaaacaccgcggtcagtgacgcagcggagttttagagctagaaat

SEQ ID NO: 2 - DNA, 54 bp, Artificial Sequence
  DNA primer
ggaaaggacgaaacaccgccttctgcaactccgacctgttttagagctagaaat

SEQ ID NO: 3 - DNA, 54 bp, Artificial Sequence
  DNA primer
ggaaaggacgaaacaccgcaagttcacgtctatccgtgttttagagctagaaat

SEQ ID NO: 4 - DNA, 54 bp, Artificial Sequence
  DNA primer
ggaaaggacgaaacaccgatctccacgcggccctcacgttttagagctagaaat

SEQ ID NO: 5 - DNA, 54 bp, Artificial Sequence
  DNA primer
ggaaaggacgaaacaccgtgactgagcctgatccggagttttagagctagaaat

SEQ ID NO: 6 - DNA, 54 bp, Artificial Sequence
  DNA primer
ggaaaggacgaaacaccgttgcggccgagatggtcaagttttagagctagaaat

SEQ ID NO: 7 - DNA, 53 bp, Artificial Sequence
  DNA primer
ctaaaactccgctgcgtcactgaccgcggtgtttcgtcctttccacaagatat

SEQ ID NO: 8 - DNA, 53 bp, Artificial Sequence
  DNA primer
ctaaaacaggtcggagttgcagaaggcggtgtttcgtcctttccacaagatat

SEQ ID NO: 9 - DNA, 53 bp, Artificial Sequence
  DNA primer
ctaaaacacggatagacgtgaacttgcggtgtttcgtcctttccacaagatat

SEQ ID NO: 10 - DNA, 53 bp, Artificial Sequence
  DNA primer
ctaaaacgtgagggccgcgtggagatcggtgtttcgtcctttccacaagatat

SEQ ID NO: 11 - DNA, 53 bp, Artificial Sequence
  DNA primer
ctaaaactccggatcaggctcagtcacggtgtttcgtcctttccacaagatat

SEQ ID NO: 12 - DNA, 53 bp, Artificial Sequence
  DNA primer
ctaaaacttgaccatctcggccgcaacggtgtttcgtcctttccacaagatat

SEQ ID NO: 13 - DNA, 22 bp, Artificial Sequence
  DNA primer
catggtggctactactgctttt

SEQ ID NO: 14 - DNA, 22 bp, Artificial Sequence
  DNA primer
tcactgataacctccagcaagg

SEQ ID NO: 15 - DNA, 22 bp, Artificial Sequence
  DNA primer
ctcagcaggtgactgattggag

SEQ ID NO: 16 - DNA, 21 bp, Artificial Sequence
  DNA primer
gcacaaagcatcgaagtcctg

SEQ ID NO: 17 - DNA, 19 bp, Artificial Sequence
  DNA primer
tgggtagggactgctaccg

SEQ ID NO: 18 - DNA, 22 bp, Artificial Sequence
  DNA primer
tgccatccattcttgcaacttc

SEQ ID NO: 19 - DNA, 20 bp, Artificial Sequence
  DNA primer
caaggtgggcatcaacgact

SEQ ID NO: 20 - DNA, 23 bp, Artificial Sequence
  DNA primer
atggccaaagtggatctatgcaa

SEQ ID NO: 21 - DNA, 22 bp, Artificial Sequence
  DNA primer
agcctggagtatccttgggtag

SEQ ID NO: 22 - DNA, 25 bp, Artificial Sequence
  DNA primer
gcatctaaaatgttccagaggttgt

SEQ ID NO: 23 - DNA, 22 bp, Artificial Sequence
  DNA primer
tggagtcatcatggacacactc

SEQ ID NO: 24 - DNA, 23 bp, Artificial Sequence
  DNA primer
tcccatttggtttctcaaggttt